European Patent Application EP 4 442 813 A1, published October 9, 2024. Title: IMMUNE CELLS WITH ENHANCED EFFICACY. Applicant: KOREA RESEARCH INSTITUTE OF CHEMICAL TECHNOLOGY. Application KR. The sequence listing filed with the application follows.

SEQUENCE LISTING (18 sequences)

SEQ ID NO: 1 - DNA, 21 bp, synthetic construct
  misc_feature 1..21: note = 1st target sequence in Tet2
  source 1..21: mol_type = other DNA
tttcacgccaagtcgttattt

SEQ ID NO: 2 - DNA, 21 bp, synthetic construct
  misc_feature 1..21: note = 2nd target sequence in Tet2
  source 1..21: mol_type = other DNA
gcacacacatgtatatgtata

SEQ ID NO: 3 - DNA, 19 bp, synthetic construct
  misc_feature 1..19: note = 3rd target sequence in Tet2
  source 1..19: mol_type = other DNA
gcaccaccagaaaacaaaa

SEQ ID NO: 4 - DNA, 19 bp, synthetic construct
  misc_feature 1..19: note = 4th target sequence in Tet2
  source 1..19: mol_type = other DNA
ggatgacccaaaagaggaa

SEQ ID NO: 5 - DNA, 19 bp, synthetic construct
  misc_feature 1..19: note = 5th target sequence in Tet2
  source 1..19: mol_type = other DNA
ggaaactagaagccaagaa

SEQ ID NO: 6 - DNA, 19 bp, synthetic construct
  misc_feature 1..19: note = 6th target sequence in Tet2
  source 1..19: mol_type = other DNA
gcaatccaaacatggacta

SEQ ID NO: 7 - DNA, 19 bp, synthetic construct
  misc_feature 1..19: note = 7th target sequence in Tet2
  source 1..19: mol_type = other DNA
gcatctaggaaaagaccaa

SEQ ID NO: 8 - DNA, 19 bp, synthetic construct
  misc_feature 1..19: note = 8th target sequence in Tet2
  source 1..19: mol_type = other DNA
gcatagtcatggaacacaa

SEQ ID NO: 9 - DNA, 21 bp, synthetic construct
  misc_feature 1..21: note = 9th target sequence in Tet2
  source 1..21: mol_type = other DNA
gaagcagtttcacgccaagtc

SEQ ID NO: 10 - DNA, 58 bp, synthetic construct
  misc_feature 1..58: note = polynucleotide sequence encoding 1st shRNA
  source 1..58: mol_type = other DNA
ccggtttcacgccaagtcgttatttgctagcaaataacgacttggcgtgaaatttttg

SEQ ID NO: 11 - DNA, 58 bp, synthetic construct
  misc_feature 1..58: note = polynucleotide sequence encoding 2nd shRNA
  source 1..58: mol_type = other DNA
ccgggcacacacatgtatatgtatagctagctatacatatacatgtgtgtgctttttg

SEQ ID NO: 12 - DNA, 54 bp, synthetic construct
  misc_feature 1..54: note = polynucleotide sequence encoding 3rd shRNA
  source 1..54: mol_type = other DNA
ccgggcaccaccagaaaacaaaagctagcttttgttttctggtggtgctttttg

SEQ ID NO: 13 - DNA, 54 bp, synthetic construct
  misc_feature 1..54: note = polynucleotide sequence encoding 4th shRNA
  source 1..54: mol_type = other DNA
ccggggatgacccaaaagaggaagctagcttcctcttttgggtcatcctttttg

SEQ ID NO: 14 - DNA, 54 bp, synthetic construct
  misc_feature 1..54: note = polynucleotide sequence encoding 5th shRNA
  source 1..54: mol_type = other DNA
ccggggaaactagaagccaagaagctagcttcttggcttctagtttcctttttg

SEQ ID NO: 15 - DNA, 54 bp, synthetic construct
  misc_feature 1..54: note = polynucleotide sequence encoding 6th shRNA
  source 1..54: mol_type = other DNA
ccgggcaatccaaacatggactagctagctagtccatgtttggattgctttttg

SEQ ID NO: 16 - DNA, 54 bp, synthetic construct
  misc_feature 1..54: note = polynucleotide sequence encoding 7th shRNA
  source 1..54: mol_type = other DNA
ccgggcatctaggaaaagaccaagctagcttggtcttttcctagatgctttttg

SEQ ID NO: 17 - DNA, 54 bp, synthetic construct
  misc_feature 1..54: note = polynucleotide sequence encoding 8th shRNA
  source 1..54: mol_type = other DNA
ccgggcatagtcatggaacacaagctagcttgtgttccatgactatgctttttg

SEQ ID NO: 18 - DNA, 58 bp, synthetic construct
  misc_feature 1..58: note = polynucleotide sequence encoding 9th shRNA
  source 1..58: mol_type = other DNA
ccgggaagcagtttcacgccaagtcgctagcgacttggcgtgaaactgcttctttttg